European Patent Application EP 4 726 391 A1, published April 15, 2026. Title: Novel citrullinated peptides that bind to anti-citrullinated protein antibodies (ACPAs) and their use in the diagnosis and prediction of rheumatoid arthritis. Applicant: Vacara AB. Application EP, filed October 10, 2024. The sequence listing filed with the application follows.

SEQUENCE LISTING (181 sequences)

SEQ ID NO: 1-2 - skipped (2 entries)

SEQ ID NO: 3 - protein, 15 aa, synthetic construct
  MOD_RES 8: note = X = Citrulline
SKAKFAGXNFRNPLA

SEQ ID NO: 4 - protein, 15 aa, synthetic construct
  MOD_RES 8: note = X = Citrulline
VSPPVTVXGKEYPLG

SEQ ID NO: 5 - protein, 14 aa, synthetic construct
  MOD_RES 8: note = X = Citrulline
VRVFQATXGKLSSK

SEQ ID NO: 6 - protein, 15 aa, synthetic construct
  MOD_RES 8: note = X = Citrulline
DFFTYHIXHGEVHCG

SEQ ID NO: 7 - protein, 15 aa, synthetic construct
  MOD_RES 8: note = X = Citrulline
EKGVPLYXHIADLAG

SEQ ID NO: 8-9 - skipped (2 entries)

SEQ ID NO: 10 - protein, 18 aa, synthetic construct
  SITE 2: note = MISC_FEATURE - X1 is S or V
  SITE 3: note = MISC_FEATURE - X2 is K or S
  SITE 4: note = MISC_FEATURE - X3 is A or P
  SITE 5: note = MISC_FEATURE - X4 is K or P
  SITE 6: note = MISC_FEATURE - X5 is F or V
  SITE 7: note = MISC_FEATURE - X6 is A or T
  SITE 8: note = MISC_FEATURE - X7 is G or V
  SITE 9: note = X = Citrulline
  SITE 10: note = MISC_FEATURE - X8 is N or G
  SITE 11: note = MISC_FEATURE - X9 is F or K
  SITE 12: note = MISC_FEATURE - X10 is R or E
  SITE 13: note = MISC_FEATURE - X11 is N orY
  SITE 16: note = MISC_FEATURE - X12 is A or G
CXXXXXXXXXXXXPLXCA

SEQ ID NO: 11 - protein, 18 aa, synthetic construct
  MOD_RES 9: note = X = Citrulline
CSKAKFAGXNFRNPLACA

SEQ ID NO: 12 - protein, 18 aa, synthetic construct
  MOD_RES 9: note = X = Citrulline
CVSPPVTVXGKEYPLGCA

SEQ ID NO: 13 - protein, 17 aa, synthetic construct
  MOD_RES 9: note = X = Citrulline
CVRVFQATXGKLSSKCA

SEQ ID NO: 14 - protein, 16 aa, synthetic construct
  MOD_RES 9: note = X = Citrulline
CDFFTYHIXHGEVHCG

SEQ ID NO: 15 - protein, 18 aa, synthetic construct
  MOD_RES 9: note = X = Citrulline
CEKGVPLYXHIADLAGCA

SEQ ID NO: 16-20 - skipped (5 entries)

SEQ ID NO: 21 - protein, 7 aa, synthetic construct
SKAKFAG

SEQ ID NO: 22 - protein, 7 aa, synthetic construct
VSPPVTV

SEQ ID NO: 23 - protein, 7 aa, synthetic construct
VRVFQAT

SEQ ID NO: 24 - protein, 7 aa, synthetic construct
DFFTYHI

SEQ ID NO: 25 - protein, 7 aa, synthetic construct
EKGVPLY

SEQ ID NO: 26 - protein, 7 aa, synthetic construct
NFRNPLA

SEQ ID NO: 27 - protein, 7 aa, synthetic construct
GKEYPLG

SEQ ID NO: 28 - protein, 6 aa, synthetic construct
GKLSSK

SEQ ID NO: 29 - protein, 7 aa, synthetic construct
HGEVHCG

SEQ ID NO: 30 - protein, 7 aa, synthetic construct
HIADLAG

SEQ ID NO: 31 - protein, 8 aa, synthetic construct
CSKAKFAG

SEQ ID NO: 32 - protein, 8 aa, synthetic construct
CVSPPVTV

SEQ ID NO: 33 - protein, 8 aa, synthetic construct
CVRVFQAT

SEQ ID NO: 34 - protein, 8 aa, synthetic construct
CDFFTYHI

SEQ ID NO: 35 - protein, 8 aa, synthetic construct
CEKGVPLY

SEQ ID NO: 36 - protein, 9 aa, synthetic construct
NFRNPLACA

SEQ ID NO: 37 - protein, 9 aa, synthetic construct
GKEYPLGCA

SEQ ID NO: 38 - protein, 8 aa, synthetic construct
GKLSSKCA

SEQ ID NO: 39 - protein, 7 aa, synthetic construct
HGEVHCG

SEQ ID NO: 40 - protein, 9 aa, synthetic construct
HIADLAGCA

SEQ ID NO: 41-42 - skipped (2 entries)

SEQ ID NO: 43 - protein, 17 aa, synthetic construct
CVRGGSLGIFGGSVGYW

SEQ ID NO: 44 - protein, 11 aa, synthetic construct
CQSYYRGDWVL

SEQ ID NO: 45 - protein, 7 aa, synthetic construct
GYNFSHF

SEQ ID NO: 46 - protein, 6 aa, synthetic construct
NTKTAN

SEQ ID NO: 47 - protein, 13 aa, synthetic construct
GGSLGIFGGSVGY

SEQ ID NO: 48 - protein, 13 aa, synthetic construct
TANGAHIGDSYVQ

SEQ ID NO: 49 - protein, 7 aa, synthetic construct
EDDKRPS

SEQ ID NO: 50 - protein, 9 aa, synthetic construct
QSYYRGDWV

SEQ ID NO: 51 - protein, 110 aa, synthetic construct
NLTLIQSRSVSGSPGQTVSISCTANGAHIGDSYVQWFQQRPGSAPRSVIFEDDKRPSGVPDRLSGSTDFSSNSASLTISGLESEDEADYYCQSYYRGDWVLGGGTKLTVL

SEQ ID NO: 52 - protein, 123 aa, synthetic construct
QVHLEQSGSELKKPGASVTISCKTSGYNFSHFAINWVRQAPGQGLQWMGWINTKTANLTYAQTFTGRFVFSFDTSVSTAYLHIHGLKTEDTAMYYCVRGGSLGIFGGSVGYWGQGALVSVSSA

SEQ ID NO: 53 - protein, 13 aa, synthetic construct
SGDDSILRSAFVS

SEQ ID NO: 54 - protein, 7 aa, synthetic construct
DDRQRPS

SEQ ID NO: 55 - protein, 11 aa, synthetic construct
AAWNGRLSAFV

SEQ ID NO: 56-59 - skipped (4 entries)

SEQ ID NO: 60 - protein, 110 aa, synthetic construct
QSVWTQPPSVSAAPGQNVTISCSGDDSILRSAFVSWYQQVPGSAPKLVIFDDRQRPSGIPARFSGSNSGTTATLDIAGLQRGDEADYYCAAWNGRLSAFVFGSGTKLTVL

SEQ ID NO: 61 - protein, 8 aa, synthetic construct
GFPMNESY

SEQ ID NO: 62 - protein, 5 aa, synthetic construct
IHTGT

SEQ ID NO: 63 - protein, 11 aa, synthetic construct
IRGGSSNWLDP

SEQ ID NO: 64-68 - skipped (5 entries)

SEQ ID NO: 69 - protein, 121 aa, synthetic construct
QVQLEESGPGLVRPSETLSLSCTVSGFPMNESYFWGWIRQSPGKGLEWLGSVIHTGTTYYRPSLESRLTIAMDPSKNQVSLSLTSVTVADSAMYYCVRIRGGSSNWLDPWGPGIVVTASSA

SEQ ID NO: 70 - protein, 8 aa, synthetic construct
GFPMSESY

SEQ ID NO: 71 - protein, 5 aa, synthetic construct
IHTGT

SEQ ID NO: 72 - protein, 11 aa, synthetic construct
IRGGSSNWLDP

SEQ ID NO: 73-77 - skipped (5 entries)

SEQ ID NO: 78 - protein, 121 aa, synthetic construct
QVQLEESGPGLVRPSETLSLSCTVSGFPMSESYFWGWIRQSPGKGLEWLGSVIHTGTTYYRPSLESRLTIAMDPSKNQVSLSLTSVTVADSAMYYCVRIRGGSSNWLDPWGPGIVVTASSA

SEQ ID NO: 79 - protein, 13 aa, synthetic construct
SGDDSILRSAFVS

SEQ ID NO: 80 - protein, 7 aa, synthetic construct
DDRQRPS

SEQ ID NO: 81 - protein, 11 aa, synthetic construct
AAWNGRLSAFV

SEQ ID NO: 82-86 - skipped (5 entries)

SEQ ID NO: 87 - protein, 110 aa, synthetic construct
QSVWTQPPSVSAAPGQKVTISCSGDDSILRSAFVSWYQQVPGSAPKLVIFDDRQRPSGIPARFSGSNSGTTATLDIAGLQRGDEADYYCAAWNGRLSAFVFGSGTKLTVL

SEQ ID NO: 88 - protein, 121 aa, synthetic construct
AVQLVESGGGLVKPGGSLRLSCTASAFNLTNFYMSWIRQAPGKGLEWISYISRTDTFTHYADSVRGRVTISRDDANNTVYLQMNSLRVDDAAVYFCARGWDGHTASLYLDVWGRGTTVAVS

SEQ ID NO: 89 - protein, 110 aa, synthetic construct
EVVLTQTPLSLSVSPGQPASISCKSTESLQHHDGKTHLCWLVQKPGQSTQLLLYEVSRRFSGVPDRFSGSGSGTDFTLNISRVEAEDVGIYYCMQGKDLLFGQGTKLEIR

SEQ ID NO: 90 - protein, 7 aa, synthetic construct
AFNLTNF

SEQ ID NO: 91 - protein, 6 aa, synthetic construct
SRTDTF

SEQ ID NO: 92 - protein, 13 aa, synthetic construct
GWDGHTASLYLDV

SEQ ID NO: 93 - protein, 16 aa, synthetic construct
KSTESLQHHDGKTHLC

SEQ ID NO: 94 - protein, 7 aa, synthetic construct
EVSRRFS

SEQ ID NO: 95 - protein, 7 aa, synthetic construct
MQGKDLL

SEQ ID NO: 96 - protein, 433 aa, Homo sapiens
MSILKIHAREIFDSRGNPTVEVDLFTSKGLFRAAVPSGASTGIYEALELRDNDKTRYMGKGVSKAVEHINKTIAPALVSKKLNVTEQEKIDKLMIEMDGTENKSKFGANAILGVSLAVCKAGAVEKGVPLYRHIADLAGNSEVILPVPAFNVINGGSHAGNKLAMQEFMILPVGAANFREAMRIGAEVYHNLKNVIKEKYGKDATNVGDEGGFAPNILENKEGLELLKTAIGKAGYTDKVVIGMDVAASEFFRSGKYDLDFKSPDDPSRYISPDQLADLYKSFIKDYPVVSIEDPFDQDWGAWQKFTASAGIQVVGDDLTVTNPKRIAKAVNEKSCNCLLLKVNQIGSVTESLQACKLAQANGWGVMVSHRSGETEDTFIADLVVGLCTGQIKTGAPCRSERLAKYNQLLRIEEELGSKAKFAGRNFRNPLAK

SEQ ID NO: 97 - protein, 663 aa, Homo sapiens
MAQGTLIRVTPEQPTHAVCVLGTLTQLDICSSAPEDCTSFSINASPGVVVDIAHGPPAKKKSTGSSTWPLDPGVEVTLTMKVASGSTGDQKVQISYYGPKTPPVKALLYLTGVEISLCADITRTGKVKPTRAVKDQRTWTWGPCGQGAILLVNCDRDNLESSAMDCEDDEVLDSEDLQDMSLMTLSTKTPKDFFTNHTLVLHVARSEMDKVRVFQATRGKLSSKCSVVLGPKWPSHYLMVPGGKHNMDFYVEALAFPDTDFPGLITLTISLLDTSNLELPEAVVFQDSVVFRVAPWIMTPNTQPPQEVYACSIFENEDFLKSVTTLAMKAKCKLTICPEEENMDDQWMQDEMEIGYIQAPHKTLPVVFDSPRNRGLKEFPIKRVMGPDFGYVTRGPQTGGISGLDSFGNLEVSPPVTVRGKEYPLGRILFGDSCYPSNDSRQMHQALQDFLSAQQVQAPVKLYSDWLSVGHVDEFLSFVPAPDRKGFRLLLASPRSCYKLFQEQQNEGHGEALLFEGIKKKKQQKIKNILSNKTLREHNSFVERCIDWNRELLKRELGLAESDIIDIPQLFKLKEFSKAEAFFPNMVNMLVLGKHLGIPKPFGPVINGRCCLEEKVCSLLEPLGLQCTFINDFFTYHIRHGEVHCGTNVRRKPFSFKWWNMVP

SEQ ID NO: 98 - protein, 18 aa, synthetic construct
  MOD_RES 1: note = CONJUGATION: Biotin-6-Aminohexanoic Acid (Ahx)
CSILKIHAREIFDSRGCA

SEQ ID NO: 99 - protein, 18 aa, synthetic construct
  MOD_RES 1: note = CONJUGATION: Biotin-6-Aminohexanoic Acid (Ahx)
CAREIFDSRGNPTVEVCA

SEQ ID NO: 100 - protein, 18 aa, synthetic construct
  MOD_RES 1: note = CONJUGATION: Biotin-6-Aminohexanoic Acid (Ahx)
CFTSKGLFRAAVPSGACA

SEQ ID NO: 101 - protein, 18 aa, synthetic construct
  MOD_RES 1: note = CONJUGATION: Biotin-6-Aminohexanoic Acid (Ahx)
CIYEALELRDNDKTRYCA

SEQ ID NO: 102 - protein, 18 aa, synthetic construct
  MOD_RES 1: note = CONJUGATION: Biotin-6-Aminohexanoic Acid (Ahx)
CLRDNDKTRYMGKGVSCA

SEQ ID NO: 103 - protein, 18 aa, synthetic construct
  MOD_RES 1: note = CONJUGATION: Biotin-6-Aminohexanoic Acid (Ahx)
CEKGVPLYRHIADLAGCA

SEQ ID NO: 104 - protein, 18 aa, synthetic construct
  MOD_RES 1: note = CONJUGATION: Biotin-6-Aminohexanoic Acid (Ahx)
CPVGAANFREAMRIGACA

SEQ ID NO: 105 - protein, 18 aa, synthetic construct
  MOD_RES 1: note = CONJUGATION: Biotin-6-Aminohexanoic Acid (Ahx)
CANFREAMRIGAEVYHCA

SEQ ID NO: 106 - protein, 18 aa, synthetic construct
  MOD_RES 1: note = CONJUGATION: Biotin-6-Aminohexanoic Acid (Ahx)
CVAASEFFRSGKYDLDCA

SEQ ID NO: 107 - protein, 18 aa, synthetic construct
  MOD_RES 1: note = CONJUGATION: Biotin-6-Aminohexanoic Acid (Ahx)
CKSPDDPSRYISPDQLCA

SEQ ID NO: 108 - protein, 18 aa, synthetic construct
  MOD_RES 1: note = CONJUGATION: Biotin-6-Aminohexanoic Acid (Ahx)
CLTVTNPKRIAKAVNECA

SEQ ID NO: 109 - protein, 18 aa, synthetic construct
  MOD_RES 1: note = CONJUGATION: Biotin-6-Aminohexanoic Acid (Ahx)
CWGVMVSHRSGETEDTCA

SEQ ID NO: 110 - protein, 18 aa, synthetic construct
  MOD_RES 1: note = CONJUGATION: Biotin-6-Aminohexanoic Acid (Ahx)
CIKTGAPSRSERLAKYCA

SEQ ID NO: 111 - protein, 18 aa, synthetic construct
  MOD_RES 1: note = CONJUGATION: Biotin-6-Aminohexanoic Acid (Ahx)
CGAPSRSERLAKYNQLCA

SEQ ID NO: 112 - protein, 18 aa, synthetic construct
  MOD_RES 1: note = CONJUGATION: Biotin-6-Aminohexanoic Acid (Ahx)
CAKYNQLLRIEEELGSCA

SEQ ID NO: 113 - protein, 18 aa, synthetic construct
  MOD_RES 1: note = CONJUGATION: Biotin-6-Aminohexanoic Acid (Ahx)
CSKAKFAGRNFRNPLACA

SEQ ID NO: 114 - protein, 18 aa, synthetic construct
  MOD_RES 1: note = CONJUGATION: Biotin-6-Aminohexanoic Acid (Ahx)
CKAKFAGRNFRNPLAKCA

SEQ ID NO: 115 - protein, 18 aa, synthetic construct
  MOD_RES 1: note = CONJUGATION: Biotin-6-Aminohexanoic Acid (Ahx)
  MOD_RES 9: note = X = Citrulline
CSILKIHAXEIFDSRGCA

SEQ ID NO: 116 - protein, 18 aa, synthetic construct
  MOD_RES 1: note = CONJUGATION: Biotin-6-Aminohexanoic Acid (Ahx)
  MOD_RES 9: note = X = Citrulline
CAREIFDSXGNPTVEVCA

SEQ ID NO: 117 - protein, 18 aa, synthetic construct
  MOD_RES 1: note = CONJUGATION: Biotin-6-Aminohexanoic Acid (Ahx)
  MOD_RES 9: note = X = Citrulline
CFTSKGLFXAAVPSGACA

SEQ ID NO: 118 - protein, 18 aa, synthetic construct
  MOD_RES 1: note = CONJUGATION: Biotin-6-Aminohexanoic Acid (Ahx)
  MOD_RES 9: note = X = Citrulline
CIYEALELXDNDKTRYCA

SEQ ID NO: 119 - protein, 18 aa, synthetic construct
  MOD_RES 1: note = CONJUGATION: Biotin-6-Aminohexanoic Acid (Ahx)
  MOD_RES 9: note = X = Citrulline
CLRDNDKTXYMGKGVSCA

SEQ ID NO: 120 - protein, 18 aa, synthetic construct
  MOD_RES 1: note = CONJUGATION: Biotin-6-Aminohexanoic Acid (Ahx)
  MOD_RES 9: note = X = Citrulline
CEKGVPLYXHIADLAGCA

SEQ ID NO: 121 - protein, 18 aa, synthetic construct
  MOD_RES 1: note = CONJUGATION: Biotin-6-Aminohexanoic Acid (Ahx)
  MOD_RES 9: note = X = Citrulline
CPVGAANFXEAMRIGACA

SEQ ID NO: 122 - protein, 18 aa, synthetic construct
  MOD_RES 1: note = CONJUGATION: Biotin-6-Aminohexanoic Acid (Ahx)
  MOD_RES 9: note = X = Citrulline
CANFREAMXIGAEVYHCA

SEQ ID NO: 123 - protein, 18 aa, synthetic construct
  MOD_RES 1: note = CONJUGATION: Biotin-6-Aminohexanoic Acid (Ahx)
  MOD_RES 9: note = X = Citrulline
CVAASEFFXSGKYDLDCA

SEQ ID NO: 124 - protein, 18 aa, synthetic construct
  MOD_RES 1: note = CONJUGATION: Biotin-6-Aminohexanoic Acid (Ahx)
  MOD_RES 9: note = X = Citrulline
CKSPDDPSXYISPDQLCA

SEQ ID NO: 125 - protein, 18 aa, synthetic construct
  MOD_RES 1: note = CONJUGATION: Biotin-6-Aminohexanoic Acid (Ahx)
  MOD_RES 9: note = X = Citrulline
CLTVTNPKXIAKAVNECA

SEQ ID NO: 126 - protein, 18 aa, synthetic construct
  MOD_RES 1: note = CONJUGATION: Biotin-6-Aminohexanoic Acid (Ahx)
  MOD_RES 9: note = X = Citrulline
CWGVMVSHXSGETEDTCA

SEQ ID NO: 127 - protein, 18 aa, synthetic construct
  MOD_RES 1: note = CONJUGATION: Biotin-6-Aminohexanoic Acid (Ahx)
  MOD_RES 9: note = X = Citrulline
CIKTGAPSXSERLAKYCA

SEQ ID NO: 128 - protein, 18 aa, synthetic construct
  MOD_RES 1: note = CONJUGATION: Biotin-6-Aminohexanoic Acid (Ahx)
  MOD_RES 9: note = X = Citrulline
CGAPSRSEXLAKYNQLCA

SEQ ID NO: 129 - protein, 18 aa, synthetic construct
  MOD_RES 1: note = CONJUGATION: Biotin-6-Aminohexanoic Acid (Ahx)
  MOD_RES 9: note = X = Citrulline
CAKYNQLLXIEEELGSCA

SEQ ID NO: 130 - protein, 18 aa, synthetic construct
  MOD_RES 1: note = CONJUGATION: Biotin-6-Aminohexanoic Acid (Ahx)
  MOD_RES 9: note = X=Citrulline
CSKAKFAGXNFRNPLACA

SEQ ID NO: 131 - protein, 18 aa, synthetic construct
  MOD_RES 1: note = CONJUGATION: Biotin-6-Aminohexanoic Acid (Ahx)
  MOD_RES 11: note = X = Citrulline
CKAKFAGRNFXNPLAKCA

SEQ ID NO: 132 - protein, 18 aa, synthetic construct
  MOD_RES 1: note = CONJUGATION: Biotin-6-Aminohexanoic Acid (Ahx)
CMAQGTLIRVTPEQPTCA

SEQ ID NO: 133 - protein, 18 aa, synthetic construct
  MOD_RES 1: note = CONJUGATION: Biotin-6-Aminohexanoic Acid (Ahx)
CSLSADITRTGKVKPTCA

SEQ ID NO: 134 - protein, 18 aa, synthetic construct
  MOD_RES 1: note = CONJUGATION: Biotin-6-Aminohexanoic Acid (Ahx)
CTGKVKPTRAVKDQRTCA

SEQ ID NO: 135 - protein, 17 aa, synthetic construct
  MOD_RES 1: note = CONJUGATION: Biotin-6-Aminohexanoic Acid (Ahx)
CTRAVKDQRTWTWGPCA

SEQ ID NO: 136 - protein, 18 aa, synthetic construct
  MOD_RES 1: note = CONJUGATION: Biotin-6-Aminohexanoic Acid (Ahx)
CTLVLHVARSEMDKVRCA

SEQ ID NO: 137 - protein, 18 aa, synthetic construct
  MOD_RES 1: note = CONJUGATION: Biotin-6-Aminohexanoic Acid (Ahx)
CRSEMDKVRVFQATRGCA

SEQ ID NO: 138 - protein, 17 aa, synthetic construct
  MOD_RES 1: note = CONJUGATION: Biotin-6-Aminohexanoic Acid (Ahx)
CVRVFQATRGKLSSKCA

SEQ ID NO: 139 - protein, 18 aa, synthetic construct
  MOD_RES 1: note = CONJUGATION: Biotin-6-Aminohexanoic Acid (Ahx)
CPVVFDSPRNRGLKEFCA

SEQ ID NO: 140 - protein, 18 aa, synthetic construct
  MOD_RES 1: note = CONJUGATION: Biotin-6-Aminohexanoic Acid (Ahx)
CVFDSPRNRGLKEFPICA

SEQ ID NO: 141 - protein, 18 aa, synthetic construct
  MOD_RES 1: note = CONJUGATION: Biotin-6-Aminohexanoic Acid (Ahx)
CLKEFPIKRVMGPDFGCA

SEQ ID NO: 142 - protein, 18 aa, synthetic construct
  MOD_RES 1: note = CONJUGATION: Biotin-6-Aminohexanoic Acid (Ahx)
CPDFGYVTRGPQTGGICA

SEQ ID NO: 143 - protein, 18 aa, synthetic construct
  MOD_RES 1: note = CONJUGATION: Biotin-6-Aminohexanoic Acid (Ahx)
CVSPPVTVRGKEYPLGCA

SEQ ID NO: 144 - protein, 17 aa, synthetic construct
  MOD_RES 1: note = CONJUGATION: Biotin-6-Aminohexanoic Acid (Ahx)
CGKEYPLGRILFGDSCA

SEQ ID NO: 145 - protein, 17 aa, synthetic construct
  MOD_RES 1: note = CONJUGATION: Biotin-6-Aminohexanoic Acid (Ahx)
CYPSNDSRQMHQALQCA

SEQ ID NO: 146 - protein, 18 aa, synthetic construct
  MOD_RES 1: note = CONJUGATION: Biotin-6-Aminohexanoic Acid (Ahx)
CSFVPAPDRKGFRLLLCA

SEQ ID NO: 147 - protein, 18 aa, synthetic construct
  MOD_RES 1: note = CONJUGATION: Biotin-6-Aminohexanoic Acid (Ahx)
CAPDRKGFRLLLASPRCA

SEQ ID NO: 148 - protein, 18 aa, synthetic construct
  MOD_RES 1: note = CONJUGATION: Biotin-6-Aminohexanoic Acid (Ahx)
CRLLLASPRSSYKLFQCA

SEQ ID NO: 149 - protein, 18 aa, synthetic construct
  MOD_RES 1: note = CONJUGATION: Biotin-6-Aminohexanoic Acid (Ahx)
CILSNKTLREHNSFVECA

SEQ ID NO: 150 - protein, 18 aa, synthetic construct
  MOD_RES 1: note = CONJUGATION: Biotin-6-Aminohexanoic Acid (Ahx)
CEHNSFVERSIDWNRECA

SEQ ID NO: 151 - protein, 18 aa, synthetic construct
  MOD_RES 1: note = CONJUGATION: Biotin-6-Aminohexanoic Acid (Ahx)
CERSIDWNRELLKRELCA

SEQ ID NO: 152 - protein, 18 aa, synthetic construct
  MOD_RES 1: note = CONJUGATION: Biotin-6-Aminohexanoic Acid (Ahx)
CWNRELLKRELGLAESCA

SEQ ID NO: 153 - protein, 16 aa, synthetic construct
  MOD_RES 1: note = CONJUGATION: Biotin-6-Aminohexanoic Acid (Ahx)
FGPVINGRSSLEEKVA

SEQ ID NO: 154 - protein, 16 aa, synthetic construct
  MOD_RES 1: note = CONJUGATION: Biotin-6-Aminohexanoic Acid (Ahx)
CDFFTYHIRHGEVHCG

SEQ ID NO: 155 - protein, 18 aa, synthetic construct
  MOD_RES 1: note = CONJUGATION: Biotin-6-Aminohexanoic Acid (Ahx)
CVHSGTNVRRKPFSFKCA

SEQ ID NO: 156 - protein, 18 aa, synthetic construct
  MOD_RES 1: note = CONJUGATION: Biotin-6-Aminohexanoic Acid (Ahx)
CHSGTNVRRKPFSFKWCA

SEQ ID NO: 157 - protein, 16 aa, synthetic construct
  MOD_RES 1: note = CONJUGATION: Biotin-6-Aminohexanoic Acid (Ahx)
  MOD_RES 8: note = X = Citrulline
MAQGTLIXVTPEQPTA

SEQ ID NO: 158 - protein, 18 aa, synthetic construct
  MOD_RES 1: note = CONJUGATION: Biotin-6-Aminohexanoic Acid (Ahx)
  MOD_RES 9: note = X = Citrulline
CSLSADITXTGKVKPTCA

SEQ ID NO: 159 - protein, 18 aa, synthetic construct
  MOD_RES 1: note = CONJUGATION: Biotin-6-Aminohexanoic Acid (Ahx)
  MOD_RES 9: note = X = Citrulline
CTGKVKPTXAVKDQRTCA

SEQ ID NO: 160 - protein, 17 aa, synthetic construct
  MOD_RES 1: note = CONJUGATION: Biotin-6-Aminohexanoic Acid (Ahx)
  MOD_RES 9: note = X = Citrulline
CTRAVKDQXTWTWGPCA

SEQ ID NO: 161 - protein, 18 aa, synthetic construct
  MOD_RES 1: note = CONJUGATION: Biotin-6-Aminohexanoic Acid (Ahx)
  MOD_RES 9: note = X = Citrulline
CTLVLHVAXSEMDKVRCA

SEQ ID NO: 162 - protein, 16 aa, synthetic construct
  MOD_RES 1: note = CONJUGATION: Biotin-6-Aminohexanoic Acid (Ahx)
  MOD_RES 8: note = X = Citrulline
RSEMDKVXVFQATRGA

SEQ ID NO: 163 - protein, 17 aa, synthetic construct
  MOD_RES 1: note = CONJUGATION: Biotin-6-Aminohexanoic Acid (Ahx)
  MOD_RES 9: note = X = Citrulline
CVRVFQATXGKLSSKCA

SEQ ID NO: 164 - protein, 18 aa, synthetic construct
  MOD_RES 1: note = CONJUGATION: Biotin-6-Aminohexanoic Acid (Ahx)
  MOD_RES 9: note = X = Citrulline
CPVVFDSPXNRGLKEFCA

SEQ ID NO: 165 - protein, 18 aa, synthetic construct
  MOD_RES 1: note = CONJUGATION: Biotin-6-Aminohexanoic Acid (Ahx)
  MOD_RES 9: note = X = Citrulline
CVFDSPRNXGLKEFPICA

SEQ ID NO: 166 - protein, 18 aa, synthetic construct
  MOD_RES 1: note = CONJUGATION: Biotin-6-Aminohexanoic Acid (Ahx)
  MOD_RES 9: note = X = Citrulline
CLKEFPIKXVMGPDFGCA

SEQ ID NO: 167 - protein, 18 aa, synthetic construct
  MOD_RES 1: note = CONJUGATION: Biotin-6-Aminohexanoic Acid (Ahx)
  MOD_RES 9: note = X = Citrulline
CPDFGYVTXGPQTGGICA

SEQ ID NO: 168 - protein, 18 aa, synthetic construct
  MOD_RES 1: note = CONJUGATION: Biotin-6-Aminohexanoic Acid (Ahx)
  MOD_RES 9: note = X = Citrulline
CVSPPVTVXGKEYPLGCA

SEQ ID NO: 169 - protein, 17 aa, synthetic construct
  MOD_RES 1: note = CONJUGATION: Biotin-6-Aminohexanoic Acid (Ahx)
  MOD_RES 9: note = X = Citrulline
CGKEYPLGXILFGDSCA

SEQ ID NO: 170 - protein, 17 aa, synthetic construct
  MOD_RES 1: note = CONJUGATION: Biotin-6-Aminohexanoic Acid (Ahx)
  MOD_RES 8: note = X = Citrulline
CYPSNDSXQMHQALQCA

SEQ ID NO: 171 - protein, 18 aa, synthetic construct
  MOD_RES 1: note = CONJUGATION: Biotin-6-Aminohexanoic Acid (Ahx)
  MOD_RES 9: note = X = Citrulline
CSFVPAPDXKGFRLLLCA

SEQ ID NO: 172 - protein, 18 aa, synthetic construct
  MOD_RES 1: note = CONJUGATION: Biotin-6-Aminohexanoic Acid (Ahx)
  MOD_RES 9: note = X = Citrulline
CAPDRKGFXLLLASPRCA

SEQ ID NO: 173 - protein, 18 aa, synthetic construct
  MOD_RES 1: note = CONJUGATION: Biotin-6-Aminohexanoic Acid (Ahx)
  MOD_RES 9: note = X = Citrulline
CRLLLASPXSSYKLFQCA

SEQ ID NO: 174 - protein, 16 aa, synthetic construct
  MOD_RES 1: note = CONJUGATION: Biotin-6-Aminohexanoic Acid (Ahx)
  MOD_RES 8: note = X = Citrulline
ILSNKTLXEHNSFVEA

SEQ ID NO: 175 - protein, 18 aa, synthetic construct
  MOD_RES 1: note = CONJUGATION: Biotin-6-Aminohexanoic Acid (Ahx)
  MOD_RES 8: note = X = Citrulline
CEHNSFVEXSIDWNRECA

SEQ ID NO: 176 - protein, 18 aa, synthetic construct
  MOD_RES 1: note = CONJUGATION: Biotin-6-Aminohexanoic Acid (Ahx)
  MOD_RES 9: note = X = Citrulline
CERSIDWNXELLKRELCA

SEQ ID NO: 177 - protein, 18 aa, synthetic construct
  MOD_RES 1: note = CONJUGATION: Biotin-6-Aminohexanoic Acid (Ahx)
  MOD_RES 9: note = X = Citrulline
CWNRELLKXELGLAESCA

SEQ ID NO: 178 - protein, 16 aa, synthetic construct
  MOD_RES 1: note = CONJUGATION: Biotin-6-Aminohexanoic Acid (Ahx)
  MOD_RES 8: note = X = Citrulline
FGPVINGXSSLEEKVA

SEQ ID NO: 179 - protein, 16 aa, synthetic construct
  MOD_RES 1: note = CONJUGATION: Biotin-6-Aminohexanoic Acid (Ahx)
  MOD_RES 9: note = X = Citrulline
CDFFTYHIXHGEVHCG

SEQ ID NO: 180 - protein, 18 aa, synthetic construct
  MOD_RES 1: note = CONJUGATION: Biotin-6-Aminohexanoic Acid (Ahx)
  MOD_RES 9: note = X = Citrulline
CVHSGTNVXRKPFSFKCA

SEQ ID NO: 181 - protein, 18 aa, synthetic construct
  MOD_RES 1: note = CONJUGATION: Biotin-6-Aminohexanoic Acid (Ahx)
  MOD_RES 9: note = X = Citrulline
CHSGTNVRXKPFSFKWCA